European Patent Application EP 4 660 203 A1, published December 10, 2025. Title: Pharmaceutical Combination of Anti-αvβ3 Antibody and Anti-PD-1 Antibody. Applicant: NEWSOARA BIOPHARMA CO., LTD. Application CN. The sequence listing filed with the application follows.

SEQUENCE LISTING (13 sequences)

SEQ ID NO: 1 - protein, 5 aa, synthetic construct
SYDMS

SEQ ID NO: 2 - protein, 17 aa, synthetic construct
KVSSGGGSTYYLDTVQG

SEQ ID NO: 3 - protein, 8 aa, synthetic construct
HLHGSFAS

SEQ ID NO: 4 - protein, 11 aa, synthetic construct
QASQSISNFLH

SEQ ID NO: 5 - protein, 7 aa, synthetic construct
YRSQSIS

SEQ ID NO: 6 - protein, 9 aa, synthetic construct
QQSGSWPLT

SEQ ID NO: 7 - protein, 117 aa, synthetic construct
QVQLVESGGGVVQPGRSLRLSCAASGFTFSSYDMSWVRQAPGKGLEWVAKVSSGGGSTYYLDTVQGRFTISRDNSKNTLYLQMNSLRAEDTAVYYCARHLHGSFASWGQGTTVTVSS

SEQ ID NO: 8 - protein, 107 aa, synthetic construct
EIVLTQSPATLSLSPGERATLSCQASQSISNFLHWYQQRPGQAPRLLIRYRSQSISGIPARFSGSGSGTDFTLTISSLEPEDFAVYYCQQSGSWPLTFGGGTKVEIK

SEQ ID NO: 9 - protein, 229 aa, synthetic construct
ESKYGPPCPPCPAPEFLGGPSVFLFPPKPKDTLMISRTPEVTCVVVDVSQEDPEVQFNWYVDGVEVHNAKTKPREEQFNSTYRVVSVLTVLHQDWLNGKEYKCKVSNKGLPSSIEKTISKAKGQPREPQVYTLPPSQEEMTKNQVSLTCLVKGFYPSDIAVEWESNGQPENNYKTTPPVLDSDGSFFLYSRLTVDKSRWQEGNVFSCSVMHEALHNHYTQKSLSLSLGK

SEQ ID NO: 10 - protein, 444 aa, synthetic construct
QVQLVESGGGVVQPGRSLRLSCAASGFTFSSYDMSWVRQAPGKGLEWVAKVSSGGGSTYYLDTVQGRFTISRDNSKNTLYLQMNSLRAEDTAVYYCARHLHGSFASWGQGTTVTVSSASTKGPSVFPLAPCSRSTSESTAALGCLVKDYFPEPVTVSWNSGALTSGVHTFPAVLQSSGLYSLSSVVTVPSSSLGTKTYTCNVDHKPSNTKVDKRVESKYGPPCPPCPAPEFLGGPSVFLFPPKPKDTLMISRTPEVTCVVVDVSQEDPEVQFNWYVDGVEVHNAKTKPREEQFNSTYRVVSVLTVLHQDWLNGKEYKCKVSNKGLPSSIEKTISKAKGQPREPQVYTLPPSQEEMTKNQVSLTCLVKGFYPSDIAVEWESNGQPENNYKTTPPVLDSDGSFFLYSRLTVDKSRWQEGNVFSCSVMHEALHNHYTQKSLSLSLGK

SEQ ID NO: 11 - protein, 214 aa, synthetic construct
EIVLTQSPATLSLSPGERATLSCQASQSISNFLHWYQQRPGQAPRLLIRYRSQSISGIPARFSGSGSGTDFTLTISSLEPEDFAVYYCQQSGSWPLTFGGGTKVEIKRTVAAPSVFIFPPSDEQLKSGTASVVCLLNNFYPREAKVQWKVDNALQSGNSQESVTEQDSKDSTYSLSSTLTLSKADYEKHKVYACEVTHQGLSSPVTKSFNRGEC

SEQ ID NO: 12 - DNA, 1332 bp, synthetic construct
  source 1..1332: mol_type = other DNA
caagtgcagctggtggaatccggcggaggagtcgtgcagcctggcagatccctgcggctgtcctgtgctgctagtggatttaccttcagctcctacgacatgtcctgggtgcggcaggctccaggaaaaggcctggaatgggtggccaaggtgtcctctggcggcggctctacctactacctggacaccgtccaaggccgcttcaccatctctcgggacaactctaagaacaccctgtatctgcagatgaactcgctgagagccgaggacaccgctgtgtactactgcgccagacacctgcacggcagcttcgcctcttggggacagggcaccaccgtgaccgtgtccagcgccagcaccaagggcccttccgtgttccctctcgccccatgctcccggtctacctccgagtctaccgctgccctgggctgcctggtgaaggactacttccccgaacctgtgacagtcagctggaactccggcgctctgacctctggcgtgcacacctttcctgccgtgctgcagtccagcggcctgtactctctgtcttccgtggtgaccgtgccttccagctctctcggcaccaagacctacacctgcaacgtggaccacaagcctagcaataccaaagtggataaaagagtggagtccaagtacggcccaccttgccctccttgtcctgctcctgagttcctgggcggaccttctgtgtttctgttccctcctaagcccaaggataccctgatgatctcccggacccctgaggtgacttgcgtggtggttgacgtgtctcaggaagatcctgaagtgcagttcaactggtacgtggatggcgtggaagtgcacaacgccaagacaaagcctagagaggaacagttcaactccacctacagagtggtctccgtgctgaccgtgctgcatcaggactggctgaacggcaaagagtacaagtgcaaggtgtccaacaagggcctgccctcttccatcgagaagacaatctccaaggccaaaggccagcctcgggagcctcaggtttatacactgcctccatctcaagaagagatgaccaagaaccaggtgtctttgacctgtctggtcaagggcttctacccctctgacatcgccgtcgagtgggagtctaatggccagcccgagaacaactacaagacaacaccccccgtgctggattccgacggctccttcttcctgtactccagactgacagtggacaagtccagatggcaggagggcaacgtgttctcctgctctgtgatgcacgaggctttgcataaccactacacccagaagtccctgagcctgagcctgggtaag

SEQ ID NO: 13 - DNA, 642 bp, synthetic construct
  source 1..642: mol_type = other DNA
gagatcgtgctgacacagtctcctgctaccctgtccctgagccccggagaacgggctacactgagctgtcaggcctctcagagcatctccaattttctgcactggtaccagcagcggccaggccaggctcctcgcctgttgatcagatatagatcccagtccatctccggcatccccgctagattctccggctctggatctggcaccgatttcaccctgaccatcagcagcctggaacctgaggacttcgccgtgtactactgccaacagagtggctcttggcctctgaccttcggcggcggaactaaagtggaaatcaagcggaccgtggccgctccttctgtgttcatctttcctcctagcgatgaacagctgaagtctggcaccgcctctgtggtctgcctgctgaacaacttctaccccagagaggccaaagtgcagtggaaggtggacaacgccctgcagtccggcaactcccaagagtccgtgaccgagcaggactccaaggactctacctactccctgtcctccaccctgacactgtctaaggccgactacgagaagcacaaggtgtacgcctgcgaggtgacccatcagggcctgtcctctcctgtgaccaagtccttcaacagaggcgagtgc